European Patent Application EP 4 424 701 A1, published September 4, 2024. Title: 一种用于有效递送核酸的环状多肽载体及其变化形式. Applicant: 苏州慧疗生物医药科技有限公司. Application CN. The sequence listing filed with the application follows.

SEQUENCE LISTING (65 sequences)

SEQ ID NO: 1 - protein, 19 aa, Synthetic Construct
AALAALCKKKKKCLAALAA

SEQ ID NO: 2 - protein, 25 aa, Synthetic Construct
AALAALAALCKKKKKCLAALAALAA

SEQ ID NO: 3 - protein, 25 aa, Synthetic Construct
KALKALKALCALKLACLAKLAKLAK

SEQ ID NO: 4 - protein, 25 aa, Synthetic Construct
AKALAKALCKKKKKKKCLAKALAKA

SEQ ID NO: 5 - protein, 25 aa, Synthetic Construct
AKALAKALCGKKKKKGCLAKALAKA

SEQ ID NO: 6 - protein, 25 aa, Synthetic Construct
AAALAAALCGKKKKKGCLAAALAAA

SEQ ID NO: 7 - protein, 25 aa, Synthetic Construct
KKMLKKMLCGKKKKKGCLMKKLMKK

SEQ ID NO: 8 - protein, 25 aa, Synthetic Construct
KKKLKKKLCALAKALACLKKKLKKK

SEQ ID NO: 9 - protein, 28 aa, Synthetic Construct
KGLKGLCKKKKKKKKKKKKKKCLGKLGK

SEQ ID NO: 10 - protein, 28 aa, Synthetic Construct
KGLKGLCGGKGGKGGKGGKGGCLGKLGK

SEQ ID NO: 11 - protein, 28 aa, Synthetic Construct
KKLKKLCKKKKKKKKKKKKKKCLKKLKK

SEQ ID NO: 12 - protein, 28 aa, Synthetic Construct
KLLKLLCKKKKKKKKKKKKKKCLLKLLK

SEQ ID NO: 13 - protein, 28 aa, Synthetic Construct
KLLKLLCLKKLKKLKKLKKKLCLLKLLK

SEQ ID NO: 14 - protein, 28 aa, Synthetic Construct
KKLKKLCAKKAKKAKKAKKKACLLKLLK

SEQ ID NO: 15 - protein, 34 aa, Synthetic Construct
KKLKKLKKLCAKKAKKAKKAKKKACLLKLLKLLK

SEQ ID NO: 16 - protein, 34 aa, Synthetic Construct
KKLKKLKKLCAFKAFKAFKAFKFACLLKLLKLLK

SEQ ID NO: 17 - protein, 28 aa, Synthetic Construct
KKLKKLKKLKKLCAFKAFKAFKAFKFAC

SEQ ID NO: 18 - protein, 25 aa, Synthetic Construct
AKLAKLAKLCAFKAFKAFKAFKFAC

SEQ ID NO: 19 - protein, 35 aa, Synthetic Construct
KKKLKKKLCALAKALAMAKAMAKAMACLKKKLKKK

SEQ ID NO: 20 - protein, 33 aa, Synthetic Construct
KKKLKKKLCAFAKAFAKAFAKAFACLKKKLKKK

SEQ ID NO: 21 - protein, 31 aa, Synthetic Construct
KLLKLLKLLKLLCKKKKKCLLKLLKLLKLLK

SEQ ID NO: 22 - protein, 39 aa, Synthetic Construct
KKKLKKKLCFGFKFGFKFGFKFGFKFGFCLKKKKLKKKK

SEQ ID NO: 23 - protein, 37 aa, Synthetic Construct
KGVLKGVLCGKKKGKKKGKKKGKKKKKGCLVGKLVGK

SEQ ID NO: 24 - protein, 41 aa, Synthetic Construct
KAMLKAMLKAMLCKKKKKKKKKKKKKKKCLMAKLMAKLMAK

SEQ ID NO: 25 - protein, 41 aa, Synthetic Construct
KAFLKAFLKAFLCKKKKKKKKKKKKKKKCLFAKLFAKLFAK

SEQ ID NO: 26 - protein, 41 aa, Synthetic Construct
AKALAKALAKALCGKKKGKKKGKKKGKKCLAKALAKALAKA

SEQ ID NO: 27 - protein, 41 aa, Synthetic Construct
AKALAKALAKALAKALAKALAKALCGKKKGKKKGKKKKKGC

SEQ ID NO: 28 - protein, 43 aa, Synthetic Construct
RDGKKKLKKKLCGLMKGLMKGLMKGLMKMLGCLKKKLKKKGDR

SEQ ID NO: 29 - protein, 43 aa, Synthetic Construct
RDGKKKLKKKLCGLIKGLIKGLIKGLIKILGCLKKKLKKKGDR

SEQ ID NO: 30 - protein, 43 aa, Synthetic Construct
RDGKVGLKVGLCGKKKGKKKGKKKGKKKKKGCLGVKLGVKGDR

SEQ ID NO: 31 - protein, 40 aa, Synthetic Construct
RDGKKKLKKKLKKKLKKKLCGLWKGLWKGLWKGLWKWLGC

SEQ ID NO: 32 - protein, 15 aa, Synthetic Construct
AAALCKKKKKCLAAA

SEQ ID NO: 33 - protein, 15 aa, Synthetic Construct
AGALCKKKKKCLAGA

SEQ ID NO: 34 - protein, 15 aa, Synthetic Construct
ARLLCKKKKKCLLRA

SEQ ID NO: 35 - protein, 15 aa, Synthetic Construct
ADALCKKKKKCLADA

SEQ ID NO: 36 - protein, 15 aa, Synthetic Construct
AAALCKRKRKCLAAA

SEQ ID NO: 37 - protein, 15 aa, Synthetic Construct
AAALCKDKDKCLAAA

SEQ ID NO: 38 - protein, 15 aa, Synthetic Construct
AAALCKGKGKCLAAA

SEQ ID NO: 39 - protein, 15 aa, Synthetic Construct
AAALCKAKAKCLAAA

SEQ ID NO: 40 - protein, 21 aa, Synthetic Construct
ALLALLCKKKKKKKCLLALLA

SEQ ID NO: 41 - protein, 21 aa, Synthetic Construct
GSLGSLCKKKKKKKCLSGLSG

SEQ ID NO: 42 - protein, 21 aa, Synthetic Construct
ARLARLCKKKKKKKCLRALRA

SEQ ID NO: 43 - protein, 21 aa, Synthetic Construct
DLLDLLCKKKKKKKCLLDLLD

SEQ ID NO: 44 - protein, 21 aa, Synthetic Construct
ALLALLCRRKKKRRCLLALLA

SEQ ID NO: 45 - protein, 21 aa, Synthetic Construct
ALLALLCEKEKEKECLLALLA

SEQ ID NO: 46 - protein, 21 aa, Synthetic Construct
ALLALLCGGKKKGGCLLALLA

SEQ ID NO: 47 - protein, 21 aa, Synthetic Construct
ALLALLCRKRKRKRCLLALLA

SEQ ID NO: 48 - protein, 41 aa, Synthetic Construct
AALLAALLAALLCKKKKKKKKKKKKKKKCLLAALLAALLAA

SEQ ID NO: 49 - protein, 41 aa, Synthetic Construct
GGLLGGLLGGLLCKKKKKKKKKKKKKKKCLLGGLLGGLLGG

SEQ ID NO: 50 - protein, 41 aa, Synthetic Construct
DALLDALLDALLCKKKKKKKKKKKKKKKCLLADLLADLLAD

SEQ ID NO: 51 - protein, 41 aa, Synthetic Construct
AALLAALLAALLCKDKDKKDKDKKDKDKCLLAALLAALLAA

SEQ ID NO: 52 - protein, 41 aa, Synthetic Construct
AALLAALLAALLCKSKSKKSKSKKSKSKCLLAALLAALLAA

SEQ ID NO: 53 - protein, 41 aa, Synthetic Construct
AALLAALLAALLCKAKAKKAKAKKAKAKCLLAALLAALLAA

SEQ ID NO: 54 - protein, 41 aa, Synthetic Construct
AALLAALLAALLCRRKRRRRKRRRRKRRCLLAALLAALLAA

SEQ ID NO: 55 - protein, 41 aa, Synthetic Construct
AARLAARLAARLCKKKKKKKKKKKKKKKCLRAALRAALRAA

SEQ ID NO: 56 - protein, 60 aa, Synthetic Construct
AGLLAGLLAGLLAGLLAGLLAGLLCKRKRKKRKRKCLLGALLGALLGALLGALLGALLGA

SEQ ID NO: 57 - protein, 60 aa, Synthetic Construct
AGLLAGLLAGLLAGLLAGLLAGLLCKGKGKKGKGKCLLGALLGALLGALLGALLGALLGA

SEQ ID NO: 58 - protein, 80 aa, Synthetic Construct
ALGGLALGGLALGGLALGGLALGGLALGGLCKSKSKSKSKKSKSKSKSKCLGGLALGGLALGGLALGGLALGGLALGGLA

SEQ ID NO: 59 - protein, 21 aa, Synthetic Construct
RGDADALCKKKKKCLADARGD

SEQ ID NO: 60 - protein, 21 aa, Synthetic Construct
RGDAAALCKDKDKCLAAARGD

SEQ ID NO: 61 - protein, 27 aa, Synthetic Construct
RGDALLALLCEKEKEKECLLALLARGD

SEQ ID NO: 62 - protein, 16 aa, Synthetic Construct
AGALCKDKRKDCLAGA

SEQ ID NO: 63 - protein, 16 aa, Synthetic Construct
ADALCKRKEKRCLADA

SEQ ID NO: 64 - protein, 23 aa, Synthetic Construct
AILAILCKKRKKEKKRCLKALKA

SEQ ID NO: 65 - protein, 22 aa, Synthetic Construct
AELVLCKGRDKGKGKGCLVKVA